European Patent Specification EP 3 218 515 B1, published April 26, 2023. Title: THERAPEUTIC AND DIAGNOSTIC METHODS FOR IL-33-MEDIATED DISORDERS. Applicant: Genentech, Inc. F. Hoffmann-La Roche AG. The sequence listing filed with the application follows.

SEQUENCE LISTING (8 sequences)

SEQ ID NO: 1 - DNA, 51 bp, Homo sapiens
  misc_feature (26)..(26): n is Ala or Gly
tcttgtatgactagatgtagtcactncagtggaaaccaacatacgaaagag

SEQ ID NO: 2 - DNA, 51 bp, Homo sapiens
  misc_feature (26)..(26): n is Ala or Gly
gctgaggcgcttcaggactccctccngcatcttatgaaagtacaggggacc

SEQ ID NO: 3 - DNA, 51 bp, Homo sapiens
  misc_feature (26)..(26): n is Ala or Cys
ggctgaggcgcttcaggactccctcnagcatcttatgaaagtacaggggac

SEQ ID NO: 4 - DNA, 51 bp, Homo sapiens
  misc_feature (26)..(26): n is Cys or Thr
attcccagaaaggcctctagtttgantcccttggctgcccagaagcaatag

SEQ ID NO: 5 - DNA, 51 bp, Homo sapiens
  misc_feature (26)..(26): n is Cys or Thr
agaaaggcctctagtttgactccctnggctgcccagaagcaatagtgcctg

SEQ ID NO: 6 - DNA, 51 bp, Homo sapiens
  misc_feature (26)..(26): n is Gly or Thr
gattttgcaggtgtgattaaattagnaattttttttagatgaagagattat

SEQ ID NO: 7 - DNA, 51 bp, Homo sapiens
  misc_feature (26)..(26): n is Gly or Thr
ccaatcttttctcatgaagacaccancatgacctcttattcttatttatat

SEQ ID NO: 8 - DNA, 51 bp, Homo sapiens
  misc_feature (26)..(26): n is Cys or Thr
aaaaattaaagaattactgttctaangggaaattttcaggtgtaaagtctg